European Patent Specification EP 3 810 171 B1, published July 9, 2025. Title: NOVEL INTERLEUKIN-15 (IL-15) FUSION PROTEINS AND USES THEREOF. Applicant: Cugene Inc. The sequence listing filed with the application follows.

SEQUENCE LISTING (65 sequences)

SEQ ID NO: 1 - protein, 162 aa, Homo sapiens
MRISKPHLRSISIQCYLCLLLNSHFLTEAGIHVFILGCFSAGLPKTEANWVNVISDLKKIEDLIQSMHIDATLYTESDVHPSCKVTAMKCFLLELQVISLESGDASIHDTVENLIILANNSLSSNGNVTESGCKECEELEEKNIKEFLQSFVHIVQMFINTS

SEQ ID NO: 2 - protein, 114 aa, Homo sapiens
NWVNVISDLKKIEDLIQSMHIDATLYTESDVHPSCKVTAMKCFLLELQVISLESGDASIHDTVENLIILANNSLSSNGNVTESGCKECEELEEKNIKEFLQSFVHIVQMFINTS

SEQ ID NO: 3 - protein, 267 aa, Homo sapiens
MAPRRARGCRTLGLPALLLLLLLRPPATRGITCPPPMSVEHADIWVKSYSLYSRERYICNSGFKRKAGTSSLTECVLNKATNVAHWTTPSLKCIRDPALVHQRPAPPSTVTTAGVTPQPESLSPSGKEPAASSPSSNNTAATTAAIVPGSQLMPSKSPSTGTTEISSHESSHGTPSQTTAKNWELTASASHQPPGVYPQGHSDTTVAISTSTVLLCGLSAVSLLACYLKSRQTPPLASVEMEAMEALPVTWGTSSRDEDLENCSHHL

SEQ ID NO: 4 - protein, 175 aa, Homo sapiens
ITCPPPMSVEHADIWVKSYSLYSRERYICNSGFKRKAGTSSLTECVLNKATNVAHWTTPSLKCIRDPALVHQRPAPPSTVTTAGVTPQPESLSPSGKEPAASSPSSNNTAATTAAIVPGSQLMPSKSPSTGTTEISSHESSHGTPSQTTAKNWELTASASHQPPGVYPQGHSDTT

SEQ ID NO: 5 - protein, 77 aa, Homo sapiens
ITCPPPMSVEHADIWVKSYSLYSRERYICNSGFKRKAGTSSLTECVLNKATNVAHWTTPSLKCIRDPALVHQRPAPP

SEQ ID NO: 6 - protein, 226 aa, Homo sapiens
DKTHTCPPCPAPEAAGAPSVFLFPPKPKDTLMISRTPEVTCVVVDVSHEDPEVKFNWYVDGVEVHNAKTKPREEQYNSTYRVVSVLTVLHQDWLNGKEYKCKVSNKALPAPIEKTISKAKGQPREPQVYTLPPSRDELTKNQVSLTCLVKGFYPSDIAVEWESNGQPENNYKTTPPVLDSDGSFFLYSKLTVDKSRWQQGNVFSCSVMHEALHNHYTQKSLSLSPG

SEQ ID NO: 7 - protein, 226 aa, Artificial
  Knob-Fc
DKTHTCPPCPAPEAAGAPSVFLFPPKPKDTLMISRTPEVTCVVVDVSHEDPEVKFNWYVDGVEVHNAKTKPREEQYNSTYRVVSVLTVLHQDWLNGKEYKCKVSNKALPAPIEKTISKAKGQPREPQVCTLPPSREEMTKNQVSLWCLVKGFYPSDIAVEWESNGQPENNYKTTPPVLDSDGSFFLYSKLTVDKSRWQQGNVFSCSVMHEALHNHYTQKSLSLSPG

SEQ ID NO: 8 - protein, 226 aa, Artificial
  Hole-Fc
DKTHTCPPCPAPEAAGAPSVFLFPPKPKDTLMISRTPEVTCVVVDVSHEDPEVKFNWYVDGVEVHNAKTKPREEQYNSTYRVVSVLTVLHQDWLNGKEYKCKVSNKALPAPIEKTISKAKGQPREPQVYTLPPCREEMTKNQVSLSCAVKGFYPSDIAVEWESNGQPENNYKTTPPVLDSDGSFFLVSKLTVDKSRWQQGNVFSCSVMHEALHNHYTQKSLSLSPG

SEQ ID NO: 9 - protein, 15 aa, Artificial
  Peptide Linker Sequence
EPKSSDKTHTSPPSP

SEQ ID NO: 10 - protein, 10 aa, Artificial
  Peptide Linker Sequence
GGGGSGGGGS

SEQ ID NO: 11 - protein, 15 aa, Artificial
  Peptide Linker Sequence
GGGGSGGGGSGGGGS

SEQ ID NO: 12 - protein, 1 aa, Artificial
  Peptide Linker Sequence
G

SEQ ID NO: 13 - protein, 355 aa, Artificial
  Hole-Fc-Linker 1-IL-15 chain
DKTHTCPPCPAPEAAGAPSVFLFPPKPKDTLMISRTPEVTCVVVDVSHEDPEVKFNWYVDGVEVHNAKTKPREEQYNSTYRVVSVLTVLHQDWLNGKEYKCKVSNKALPAPIEKTISKAKGQPREPQVYTLPPCREEMTKNQVSLSCAVKGFYPSDIAVEWESNGQPENNYKTTPPVLDSDGSFFLVSKLTVDKSRWQQGNVFSCSVMHEALHNHYTQKSLSLSPGEPKSSDKTHTSPPSPNWVNVISDLKKIEDLIQSMHIDATLYTESDVHPSCKVTAMKCFLLELQVISLESGDASIHDTVENLIILANNSLSSNGNVTESGCKECEELEEKNIKEFLQSFVHIVQMFINTS

SEQ ID NO: 14 - protein, 318 aa, Artificial
  Knob-Fc-IL-Linker1-IL-15R??-Sushi+ chain
DKTHTCPPCPAPEAAGAPSVFLFPPKPKDTLMISRTPEVTCVVVDVSHEDPEVKFNWYVDGVEVHNAKTKPREEQYNSTYRVVSVLTVLHQDWLNGKEYKCKVSNKALPAPIEKTISKAKGQPREPQVCTLPPSREEMTKNQVSLWCLVKGFYPSDIAVEWESNGQPENNYKTTPPVLDSDGSFFLYSKLTVDKSRWQQGNVFSCSVMHEALHNHYTQKSLSLSPGEPKSSDKTHTSPPSPITCPPPMSVEHADIWVKSYSLYSRERYICNSGFKRKAGTSSLTECVLNKATNVAHWTTPSLKCIRDPALVHQRPAPP

SEQ ID NO: 15 - protein, 336 aa, Artificial
  IL-15-Linker 4-Hole-Fc chain
NWVNVISDLKKIEDLIQSMHIDATLYTESDVHPSCKVTAMKCFLLELQVISLESGDASIHDTVENLIILANNSLSSNGNVTESGCKECEELEEKNIKEFLQSFVHIVQMFINTSGCPPCPAPEAAGAPSVFLFPPKPKDTLMISRTPEVTCVVVDVSHEDPEVKFNWYVDGVEVHNAKTKPREEQYNSTYRVVSVLTVLHQDWLNGKEYKCKVSNKALPAPIEKTISKAKGQPREPQVYTLPPCREEMTKNQVSLSCAVKGFYPSDIAVEWESNGQPENNYKTTPPVLDSDGSFFLVSKLTVDKSRWQQGNVFSCSVMHEALHNHYTQKSLSLSPG

SEQ ID NO: 16 - protein, 299 aa, Artificial
  IL-15R??-Sushi+-Linker 4-Knob-Fc chain
ITCPPPMSVEHADIWVKSYSLYSRERYICNSGFKRKAGTSSLTECVLNKATNVAHWTTPSLKCIRDPALVHQRPAPPGCPPCPAPEAAGAPSVFLFPPKPKDTLMISRTPEVTCVVVDVSHEDPEVKFNWYVDGVEVHNAKTKPREEQYNSTYRVVSVLTVLHQDWLNGKEYKCKVSNKALPAPIEKTISKAKGQPREPQVCTLPPSREEMTKNQVSLWCLVKGFYPSDIAVEWESNGQPENNYKTTPPVLDSDGSFFLYSKLTVDKSRWQQGNVFSCSVMHEALHNHYTQKSLSLSPG

SEQ ID NO: 17 - protein, 313 aa, Artificial
  Knob-Fc-linker 2-IL-15R??-+ chain
DKTHTCPPCPAPEAAGAPSVFLFPPKPKDTLMISRTPEVTCVVVDVSHEDPEVKFNWYVDGVEVHNAKTKPREEQYNSTYRVVSVLTVLHQDWLNGKEYKCKVSNKALPAPIEKTISKAKGQPREPQVCTLPPSREEMTKNQVSLWCLVKGFYPSDIAVEWESNGQPENNYKTTPPVLDSDGSFFLYSKLTVDKSRWQQGNVFSCSVMHEALHNHYTQKSLSLSPGGGGGSGGGGSITCPPPMSVEHADIWVKSYSLYSRERYICNSGFKRKAGTSSLTECVLNKATNVAHWTTPSLKCIRDPALVHQRPAPP

SEQ ID NO: 18 - protein, 350 aa, Artificial
  Hole-Fc-Linker 2-IL-15 chain
DKTHTCPPCPAPEAAGAPSVFLFPPKPKDTLMISRTPEVTCVVVDVSHEDPEVKFNWYVDGVEVHNAKTKPREEQYNSTYRVVSVLTVLHQDWLNGKEYKCKVSNKALPAPIEKTISKAKGQPREPQVYTLPPCREEMTKNQVSLSCAVKGFYPSDIAVEWESNGQPENNYKTTPPVLDSDGSFFLVSKLTVDKSRWQQGNVFSCSVMHEALHNHYTQKSLSLSPGGGGGSGGGGSNWVNVISDLKKIEDLIQSMHIDATLYTESDVHPSCKVTAMKCFLLELQVISLESGDASIHDTVENLIILANNSLSSNGNVTESGCKECEELEEKNIKEFLQSFVHIVQMFINTS

SEQ ID NO: 19 - protein, 350 aa, Artificial
  IL-15-Linker 3-Hole-Fc chain
NWVNVISDLKKIEDLIQSMHIDATLYTESDVHPSCKVTAMKCFLLELQVISLESGDASIHDTVENLIILANNSLSSNGNVTESGCKECEELEEKNIKEFLQSFVHIVQMFINTSGGGGSGGGGSGGGGSCPPCPAPEAAGAPSVFLFPPKPKDTLMISRTPEVTCVVVDVSHEDPEVKFNWYVDGVEVHNAKTKPREEQYNSTYRVVSVLTVLHQDWLNGKEYKCKVSNKALPAPIEKTISKAKGQPREPQVYTLPPCREEMTKNQVSLSCAVKGFYPSDIAVEWESNGQPENNYKTTPPVLDSDGSFFLVSKLTVDKSRWQQGNVFSCSVMHEALHNHYTQKSLSLSPG

SEQ ID NO: 20 - protein, 355 aa, Artificial
  Fc-Linker 3-IL-15 chain
DKTHTCPPCPAPEAAGAPSVFLFPPKPKDTLMISRTPEVTCVVVDVSHEDPEVKFNWYVDGVEVHNAKTKPREEQYNSTYRVVSVLTVLHQDWLNGKEYKCKVSNKALPAPIEKTISKAKGQPREPQVYTLPPSRDELTKNQVSLTCLVKGFYPSDIAVEWESNGQPENNYKTTPPVLDSDGSFFLYSKLTVDKSRWQQGNVFSCSVMHEALHNHYTQKSLSLSPGGGGGSGGGGSGGGGSNWVNVISDLKKIEDLIQSMHIDATLYTESDVHPSCKVTAMKCFLLELQVISLESGDASIHDTVENLIILANNSLSSNGNVTESGCKECEELEEKNIKEFLQSFVHIVQMFINTS

SEQ ID NO: 21 - protein, 350 aa, Artificial
  IL-15-Linker 3-Fc chain
NWVNVISDLKKIEDLIQSMHIDATLYTESDVHPSCKVTAMKCFLLELQVISLESGDASIHDTVENLIILANNSLSSNGNVTESGCKECEELEEKNIKEFLQSFVHIVQMFINTSGGGGSGGGGSGGGGSCPPCPAPEAAGAPSVFLFPPKPKDTLMISRTPEVTCVVVDVSHEDPEVKFNWYVDGVEVHNAKTKPREEQYNSTYRVVSVLTVLHQDWLNGKEYKCKVSNKALPAPIEKTISKAKGQPREPQVYTLPPSRDELTKNQVSLTCAVKGFYPSDIAVEWESNGQPENNYKTTPPVLDSDGSFFLVSKLTVDKSRWQQGNVFSCSVMHEALHNHYTQKSLSLSPG

SEQ ID NO: 22 - protein, 313 aa, Artificial; identical to SEQ ID NO: 17
  Knob-Fc-Linker 2-IL-15R??-Sushi+ chain

SEQ ID NO: 23 - protein, 313 aa, Artificial
  Fc-Linker 2-IL-15R??-Sushi+ chain
DKTHTCPPCPAPEAAGAPSVFLFPPKPKDTLMISRTPEVTCVVVDVSHEDPEVKFNWYVDGVEVHNAKTKPREEQYNSTYRVVSVLTVLHQDWLNGKEYKCKVSNKALPAPIEKTISKAKGQPREPQVYTLPPSRDELTKNQVSLTCLVKGFYPSDIAVEWESNGQPENNYKTTPPVLDSDGSFFLYSKLTVDKSRWQQGNVFSCSVMHEALHNHYTQKSLSLSPGGGGGSGGGGSITCPPPMSVEHADIWVKSYSLYSRERYICNSGFKRKAGTSSLTECVLNKATNVAHWTTPSLKCIRDPALVHQRPAPP

SEQ ID NO: 24 - protein, 114 aa, Artificial
  IL-15 S58D Variant Polypeptide
NWVNVISDLKKIEDLIQSMHIDATLYTESDVHPSCKVTAMKCFLLELQVISLESGDADIHDTVENLIILANNSLSSNGNVTESGCKECEELEEKNIKEFLQSFVHIVQMFINTS

SEQ ID NO: 25 - protein, 114 aa, Artificial
  IL-15 T62D Variant Polypeptide
NWVNVISDLKKIEDLIQSMHIDATLYTESDVHPSCKVTAMKCFLLELQVISLESGDASIHDDVENLIILANNSLSSNGNVTESGCKECEELEEKNIKEFLQSFVHIVQMFINTS

SEQ ID NO: 26 - protein, 114 aa, Artificial
  IL-15 V63F Variant Polypeptide
NWVNVISDLKKIEDLIQSMHIDATLYTESDVHPSCKVTAMKCFLLELQVISLESGDASIHDTFENLIILANNSLSSNGNVTESGCKECEELEEKNIKEFLQSFVHIVQMFINTS

SEQ ID NO: 27 - protein, 114 aa, Artificial
  IL-15 I67V Variant Polypeptide
NWVNVISDLKKIEDLIQSMHIDATLYTESDVHPSCKVTAMKCFLLELQVISLESGDASIHDTVENLVILANNSLSSNGNVTESGCKECEELEEKNIKEFLQSFVHIVQMFINTS

SEQ ID NO: 28 - protein, 114 aa, Artificial
  IL-15 I68F Variant Polypeptide
NWVNVISDLKKIEDLIQSMHIDATLYTESDVHPSCKVTAMKCFLLELQVISLESGDASIHDTVENLIFLANNSLSSNGNVTESGCKECEELEEKNIKEFLQSFVHIVQMFINTS

SEQ ID NO: 29 - protein, 114 aa, Artificial
  IL-15 I68K Variant Polypeptide
NWVNVISDLKKIEDLIQSMHIDATLYTESDVHPSCKVTAMKCFLLELQVISLESGDASIHDTVENLIKLANNSLSSNGNVTESGCKECEELEEKNIKEFLQSFVHIVQMFINTS

SEQ ID NO: 30 - protein, 114 aa, Artificial
  IL-15 I68D Variant Polypeptide
NWVNVISDLKKIEDLIQSMHIDATLYTESDVHPSCKVTAMKCFLLELQVISLESGDASIHDTVENLIDLANNSLSSNGNVTESGCKECEELEEKNIKEFLQSFVHIVQMFINTS

SEQ ID NO: 31 - protein, 114 aa, Artificial
  IL-15 I68H Variant Polypeptide
NWVNVISDLKKIEDLIQSMHIDATLYTESDVHPSCKVTAMKCFLLELQVISLESGDASIHDTVENLIHLANNSLSSNGNVTESGCKECEELEEKNIKEFLQSFVHIVQMFINTS

SEQ ID NO: 32 - protein, 114 aa, Artificial
  IL-15 Q108A Variant Polypeptide
NWVNVISDLKKIEDLIQSMHIDATLYTESDVHPSCKVTAMKCFLLELQVISLESGDASIHDTVENLIILANNSLSSNGNVTESGCKECEELEEKNIKEFLQSFVHIVAMFINTS

SEQ ID NO: 33 - protein, 114 aa, Artificial
  IL-15 Q108M Variant Polypeptide
NWVNVISDLKKIEDLIQSMHIDATLYTESDVHPSCKVTAMKCFLLELQVISLESGDASIHDTVENLIILANNSLSSNGNVTESGCKECEELEEKNIKEFLQSFVHIVMMFINTS

SEQ ID NO: 34 - protein, 114 aa, Artificial
  IL-15 Q108S Variant Polypeptide
NWVNVISDLKKIEDLIQSMHIDATLYTESDVHPSCKVTAMKCFLLELQVISLESGDASIHDTVENLIILANNSLSSNGNVTESGCKECEELEEKNIKEFLQSFVHIVSMFINTS

SEQ ID NO: 35 - protein, 114 aa, Artificial
  IL-15 Q108S/D30T Variant Polypeptide
NWVNVISDLKKIEDLIQSMHIDATLYTESTVHPSCKVTAMKCFLLELQVISLESGDASIHDTVENLIILANNSLSSNGNVTESGCKECEELEEKNIKEFLQSFVHIVSMFINTS

SEQ ID NO: 36 - protein, 114 aa, Artificial
  IL-15 Q108S/V31Y Variant Polypeptide
NWVNVISDLKKIEDLIQSMHIDATLYTESDYHPSCKVTAMKCFLLELQVISLESGDASIHDTVENLIILANNSLSSNGNVTESGCKECEELEEKNIKEFLQSFVHIVSMFINTS

SEQ ID NO: 37 - protein, 114 aa, Artificial
  IL-15 Q108S/H32E Variant Polypeptide
NWVNVISDLKKIEDLIQSMHIDATLYTESDVEPSCKVTAMKCFLLELQVISLESGDASIHDTVENLIILANNSLSSNGNVTESGCKECEELEEKNIKEFLQSFVHIVSMFINTS

SEQ ID NO: 38 - protein, 114 aa, Artificial
  IL-15 Q108S/D30T/V31Y/H32E Variant Polypeptide
NWVNVISDLKKIEDLIQSMHIDATLYTESTYEPSCKVTAMKCFLLELQVISLESGDASIHDTVENLIILANNSLSSNGNVTESGCKECEELEEKNIKEFLQSFVHIVSMFINTS

SEQ ID NO: 39 - protein, 110 aa, Artificial
  IL-15 deletion 111-114 Variant Polypeptide
NWVNVISDLKKIEDLIQSMHIDATLYTESDVHPSCKVTAMKCFLLELQVISLESGDASIHDTVENLIILANNSLSSNGNVTESGCKECEELEEKNIKEFLQSFVHIVQMF

SEQ ID NO: 40 - protein, 108 aa, Artificial
  IL-15 deletion 109-114 Variant Polypeptide
NWVNVISDLKKIEDLIQSMHIDATLYTESDVHPSCKVTAMKCFLLELQVISLESGDASIHDTVENLIILANNSLSSNGNVTESGCKECEELEEKNIKEFLQSFVHIVQ

SEQ ID NO: 41 - protein, 107 aa, Artificial
  IL-15 deletion 108-114 Variant Polypeptide
NWVNVISDLKKIEDLIQSMHIDATLYTESDVHPSCKVTAMKCFLLELQVISLESGDASIHDTVENLIILANNSLSSNGNVTESGCKECEELEEKNIKEFLQSFVHIV

SEQ ID NO: 42 - protein, 104 aa, Artificial
  IL-15 deletion 105-114 Variant Polypeptide
NWVNVISDLKKIEDLIQSMHIDATLYTESDVHPSCKVTAMKCFLLELQVISLESGDASIHDTVENLIILANNSLSSNGNVTESGCKECEELEEKNIKEFLQSFV

SEQ ID NO: 43 - protein, 116 aa, Artificial
  IL-15 Insertion 'GS' after N95 Variant Polypeptide
NWVNVISDLKKIEDLIQSMHIDATLYTESDVHPSCKVTAMKCFLLELQVISLESGDASIHDTVENLIILANNSLSSNGNVTESGCKECEELEEKNGSIKEFLQSFVHIVQMFINTS

SEQ ID NO: 44 - protein, 119 aa, Artificial
  IL-15 Insertion 'GGSGG' after N95 Variant Polypeptide
NWVNVISDLKKIEDLIQSMHIDATLYTESDVHPSCKVTAMKCFLLELQVISLESGDASIHDTVENLIILANNSLSSNGNVTESGCKECEELEEKNGGSGGIKEFLQSFVHIVQMFINTS

SEQ ID NO: 45 - protein, 123 aa, Artificial
  IL-15 Insertion 'GSSGGSGGS' after N95 Variant Polypeptide
NWVNVISDLKKIEDLIQSMHIDATLYTESDVHPSCKVTAMKCFLLELQVISLESGDASIHDTVENLIILANNSLSSNGNVTESGCKECEELEEKNGSSGSSGGSIKEFLQSFVHIVQMFINTS

SEQ ID NO: 46 - protein, 355 aa, Artificial
  Fc-Linker 3-IL-15 S58D chain
DKTHTCPPCPAPEAAGAPSVFLFPPKPKDTLMISRTPEVTCVVVDVSHEDPEVKFNWYVDGVEVHNAKTKPREEQYNSTYRVVSVLTVLHQDWLNGKEYKCKVSNKALPAPIEKTISKAKGQPREPQVYTLPPSRDELTKNQVSLTCLVKGFYPSDIAVEWESNGQPENNYKTTPPVLDSDGSFFLYSKLTVDKSRWQQGNVFSCSVMHEALHNHYTQKSLSLSPGGGGGSGGGGSGGGGSNWVNVISDLKKIEDLIQSMHIDATLYTESDVHPSCKVTAMKCFLLELQVISLESGDADIHDTVENLIILANNSLSSNGNVTESGCKECEELEEKNIKEFLQSFVHIVQMFINTS

SEQ ID NO: 47 - protein, 9 aa, Artificial
  Peptide Linker Sequence
GGGGSGGGG

SEQ ID NO: 48 - protein, 355 aa, Artificial
  Hole-Fc-Linker 3-IL-15 S58D chain
DKTHTCPPCPAPEAAGAPSVFLFPPKPKDTLMISRTPEVTCVVVDVSHEDPEVKFNWYVDGVEVHNAKTKPREEQYNSTYRVVSVLTVLHQDWLNGKEYKCKVSNKALPAPIEKTISKAKGQPREPQVYTLPPCREEMTKNQVSLSCAVKGFYPSDIAVEWESNGQPENNYKTTPPVLDSDGSFFLVSKLTVDKSRWQQGNVFSCSVMHEALHNHYTQKSLSLSPGGGGGSGGGGSGGGGSNWVNVISDLKKIEDLIQSMHIDATLYTESDVHPSCKVTAMKCFLLELQVISLESGDADIHDTVENLIILANNSLSSNGNVTESGCKECEELEEKNIKEFLQSFVHIVQMFINTS

SEQ ID NO: 49 - protein, 350 aa, Artificial
  IL-15 S58D-Linker 3-Hole-Fc chain
NWVNVISDLKKIEDLIQSMHIDATLYTESDVHPSCKVTAMKCFLLELQVISLESGDADIHDTVENLIILANNSLSSNGNVTESGCKECEELEEKNIKEFLQSFVHIVQMFINTSGGGGSGGGGSGGGGSCPPCPAPEAAGAPSVFLFPPKPKDTLMISRTPEVTCVVVDVSHEDPEVKFNWYVDGVEVHNAKTKPREEQYNSTYRVVSVLTVLHQDWLNGKEYKCKVSNKALPAPIEKTISKAKGQPREPQVYTLPPCREEMTKNQVSLSCAVKGFYPSDIAVEWESNGQPENNYKTTPPVLDSDGSFFLVSKLTVDKSRWQQGNVFSCSVMHEALHNHYTQKSLSLSPG

SEQ ID NO: 50 - protein, 350 aa, Artificial
  IL-15 S58D-Linker 3-Fc chain
NWVNVISDLKKIEDLIQSMHIDATLYTESDVHPSCKVTAMKCFLLELQVISLESGDADIHDTVENLIILANNSLSSNGNVTESGCKECEELEEKNIKEFLQSFVHIVQMFINTSGGGGSGGGGSGGGGSCPPCPAPEAAGAPSVFLFPPKPKDTLMISRTPEVTCVVVDVSHEDPEVKFNWYVDGVEVHNAKTKPREEQYNSTYRVVSVLTVLHQDWLNGKEYKCKVSNKALPAPIEKTISKAKGQPREPQVYTLPPSRDELTKNQVSLTCAVKGFYPSDIAVEWESNGQPENNYKTTPPVLDSDGSFFLVSKLTVDKSRWQQGNVFSCSVMHEALHNHYTQKSLSLSPG

SEQ ID NO: 51 - protein, 308 aa, Artificial
  IL-15R??-Sushi+Linker 2-Knob-Fc chain
ITCPPPMSVEHADIWVKSYSLYSRERYICNSGFKRKAGTSSLTECVLNKATNVAHWTTPSLKCIRDPALVHQRPAPPGGGGSGGGGSCPPCPAPEAAGAPSVFLFPPKPKDTLMISRTPEVTCVVVDVSHEDPEVKFNWYVDGVEVHNAKTKPREEQYNSTYRVVSVLTVLHQDWLNGKEYKCKVSNKALPAPIEKTISKAKGQPREPQVCTLPPSREEMTKNQVSLWCLVKGFYPSDIAVEWESNGQPENNYKTTPPVLDSDGSFFLYSKLTVDKSRWQQGNVFSCSVMHEALHNHYTQKSLSLSPG

SEQ ID NO: 52 - protein, 308 aa, Artificial
  IL-15R??-Sushi+Linker 2-Fc chain
ITCPPPMSVEHADIWVKSYSLYSRERYICNSGFKRKAGTSSLTECVLNKATNVAHWTTPSLKCIRDPALVHQRPAPPGGGGSGGGGSCPPCPAPEAAGAPSVFLFPPKPKDTLMISRTPEVTCVVVDVSHEDPEVKFNWYVDGVEVHNAKTKPREEQYNSTYRVVSVLTVLHQDWLNGKEYKCKVSNKALPAPIEKTISKAKGQPREPQVYTLPPSRDELTKNQVSLTCLVKGFYPSDIAVEWESNGQPENNYKTTPPVLDSDGSFFLYSKLTVDKSRWQQGNVFSCSVMHEALHNHYTQKSLSLSPG

SEQ ID NO: 53 - protein, 355 aa, Artificial
  Hole-Fc-Linker 1-IL-15-S58D chain
DKTHTCPPCPAPEAAGAPSVFLFPPKPKDTLMISRTPEVTCVVVDVSHEDPEVKFNWYVDGVEVHNAKTKPREEQYNSTYRVVSVLTVLHQDWLNGKEYKCKVSNKALPAPIEKTISKAKGQPREPQVYTLPPCREEMTKNQVSLSCAVKGFYPSDIAVEWESNGQPENNYKTTPPVLDSDGSFFLVSKLTVDKSRWQQGNVFSCSVMHEALHNHYTQKSLSLSPGEPKSSDKTHTSPPSPNWVNVISDLKKIEDLIQSMHIDATLYTESDVHPSCKVTAMKCFLLELQVISLESGDADIHDTVENLIILANNSLSSNGNVTESGCKECEELEEKNIKEFLQSFVHIVQMFINTS

SEQ ID NO: 54 - protein, 355 aa, Artificial
  Hole-Fc-Linker 3-IL-15 chain
DKTHTCPPCPAPEAAGAPSVFLFPPKPKDTLMISRTPEVTCVVVDVSHEDPEVKFNWYVDGVEVHNAKTKPREEQYNSTYRVVSVLTVLHQDWLNGKEYKCKVSNKALPAPIEKTISKAKGQPREPQVYTLPPCREEMTKNQVSLSCAVKGFYPSDIAVEWESNGQPENNYKTTPPVLDSDGSFFLVSKLTVDKSRWQQGNVFSCSVMHEALHNHYTQKSLSLSPGGGGGSGGGGSGGGGSNWVNVISDLKKIEDLIQSMHIDATLYTESDVHPSCKVTAMKCFLLELQVISLESGDASIHDTVENLIILANNSLSSNGNVTESGCKECEELEEKNIKEFLQSFVHIVQMFINTS

SEQ ID NO: 55 - protein, 355 aa, Artificial
  Knob-Fc-Linker 1-IL-15 chain
DKTHTCPPCPAPEAAGAPSVFLFPPKPKDTLMISRTPEVTCVVVDVSHEDPEVKFNWYVDGVEVHNAKTKPREEQYNSTYRVVSVLTVLHQDWLNGKEYKCKVSNKALPAPIEKTISKAKGQPREPQVCTLPPSREEMTKNQVSLWCLVKGFYPSDIAVEWESNGQPENNYKTTPPVLDSDGSFFLYSKLTVDKSRWQQGNVFSCSVMHEALHNHYTQKSLSLSPGEPKSSDKTHTSPPSPNWVNVISDLKKIEDLIQSMHIDATLYTESDVHPSCKVTAMKCFLLELQVISLESGDASIHDTVENLIILANNSLSSNGNVTESGCKECEELEEKNIKEFLQSFVHIVQMFINTS

SEQ ID NO: 56 - DNA, 1131 bp, Artificial
  P-0313 Chain 1
atggatatgcgggtgcctgctcagctgctgggcctgctgctgctgtggctgcgaggggctagatgtgataaaactcatacttgtcctccatgcccagcacctgaggcagcaggcgccccatccgtgttcctgtttccccctaagcccaaggacacactgatgatctcccgtacgccagaggtgacatgcgtggtggtggacgtgagccacgaggaccccgaggtgaagtttaactggtacgtggacggcgtggaggtgcacaatgccaagacaaagcctagggaggagcagtacaattctacctatcgcgtggtgagcgtgctgacagtgctgcaccaggattggctgaacggcaaggagtataagtgcaaggtgtccaataaggccctgcctgccccaatcgagaagaccatctctaaggccaagggccagcccagagagcctcaggtgtacacactgcctccaagcagagacgagctgaccaagaaccaggtgtccctgacatgtctggtgaagggcttctatccctctgatatcgccgtggagtgggagagcaatggccagcctgagaacaattacaagaccacaccccctgtgctggacagcgatggctccttctttctgtattccaagctgaccgtggataagtctcggtggcagcagggcaacgtgttttcctgctctgtgatgcacgaagcactgcataaccactacacccagaagagcctgagcctgtcccccgggggaggcggaggatctggtggcggaggaagcggaggcggcggctccaactgggtgaatgtgatcagcgacctgaagaagatcgaggatctgatccagtccatgcacatcgacgccaccctgtatacagagtctgatgtgcaccccagctgcaaggtgaccgccatgaagtgttttctgctggagctgcaggtcatcagcctggagtccggcgacgcagacatccacgataccgtggagaatctgatcatcctggccaacaattccctgtctagcaacggcaatgtgacagagtctggctgcaaggagtgtgaggagctggaggagaagaatatcaaagagttcctgcagagtttcgtccacatcgtccagatgtttatcaatacctca

SEQ ID NO: 57 - DNA, 321 bp, Artificial
  Chain 2 of fusion proteins P-0313, P-0234, P-0666, and P-0668
atggctccacggcgggctcggggctgtcgcaccctggggctgcctgctctgctgctgctgctgctgctgagaccacctgctacacgcggcatcacctgcccacctccaatgagcgtggagcacgcagacatctgggtgaagtcttacagcctgtatagccgggagagatacatctgcaactccggcttcaagcggaaggccggcaccagctccctgacagagtgcgtgctgaacaaggccacaaatgtggcccactggaccacaccttccctgaagtgcatccgggaccccgccctggtgcaccagcgcccagccccccct

SEQ ID NO: 58 - DNA, 1131 bp, Artificial
  P-0234 Chain 1
atggatatgcgggtgcctgctcagctgctgggcctgctgctgctgtggctgcgaggggctagatgtgataaaactcatacttgtcctccatgcccagcacctgaggcagcaggcgccccatccgtgttcctgtttccccctaagcccaaggacacactgatgatctcccgtacgccagaggtgacatgcgtggtggtggacgtgagccacgaggaccccgaggtgaagtttaactggtacgtggacggcgtggaggtgcacaatgccaagacaaagcctagggaggagcagtacaattctacctatcgcgtggtgagcgtgctgacagtgctgcaccaggattggctgaacggcaaggagtataagtgcaaggtgtccaataaggccctgcctgccccaatcgagaagaccatctctaaggccaagggccagcccagagagcctcaggtgtacacactgcctccaagcagagacgagctgaccaagaaccaggtgtccctgacatgtctggtgaagggcttctatccctctgatatcgccgtggagtgggagagcaatggccagcctgagaacaattacaagaccacaccccctgtgctggacagcgatggctccttctttctgtattccaagctgaccgtggataagtctcggtggcagcagggcaacgtgttttcctgctctgtgatgcacgaagcactgcataaccactacacccagaagagcctgagcctgtcccccgggggaggcggaggatctggtggcggaggaagcggaggcggcggctccaactgggtgaatgtgatcagcgacctgaagaagatcgaggatctgatccagtccatgcacatcgacgccaccctgtatacagagtctgatgtgcaccccagctgcaaggtgaccgccatgaagtgttttctgctggagctgcaggtcatcagcctggagtccggcgacgcaagcatccacgataccgtggagaatctgatcatcctggccaacaattccctgtctagcaacggcaatgtgacagagtctggctgcaaggagtgtgaggagctggaggagaagaatatcaaagagttcctgcagagtttcgtccacatcgtccagatgtttatcaatacctca

SEQ ID NO: 59 - DNA, 1131 bp, Artificial
  P-0666 Chain 1
atggatatgcgagtgcctgctcagctgctgggcctgctgctgctgtggctgcggggggctagatgcgataaaactcatacctgtcctccatgcccagcacctgaggcagcaggcgccccatccgtgttcctgtttccccctaagcccaaggacaccctgatgatctctcgtacgcccgaggtgacatgcgtggtggtggacgtgagccacgaggaccccgaggtgaagttcaactggtacgtggatggcgtggaggtgcacaatgccaagacaaagcctcgggaggagcagtacaactccacctatagagtggtgtctgtgctgacagtgctgcaccaggactggctgaacggcaaggagtacaagtgcaaggtgtccaataaggccctgccagcccccatcgagaagaccatcagcaaggccaagggccagcctagggagccacaggtgtataccctgccaccctgccgcgaggagatgacaaagaaccaggtgtccctgtcttgtgccgtgaagggcttctacccttctgacatcgccgtggagtgggagagcaatggccagccagagaacaattataagaccacacctccagtgctggactctgatggcagcttctttctggtgagcaagctgaccgtggataagtccaggtggcagcagggcaacgtgtttagctgttccgtgatgcacgaggccctgcacaatcactacacacagaagtctctgagcctgtcccccgggggaggcggaggatctggtggcggaggaagcggaggcggcggctccaactgggtgaatgtgatcagcgacctgaagaagatcgaggatctgatccagtccatgcacatcgacgccaccctgtatacagagtctgatgtgcaccccagctgcaaggtgaccgccatgaagtgttttctgctggagctgcaggtcatcagcctggagtccggcgacgcagacatccacgataccgtggagaatctgatcatcctggccaacaattccctgtctagcaacggcaatgtgacagagtctggctgcaaggagtgtgaggagctggaggagaagaatatcaaagagttcctgcagagtttcgtccacatcgtccagatgtttatcaatacctca

SEQ ID NO: 60 - DNA, 744 bp, Artificial
  P-0666 Chain 3
atggatatgcgggtgcctgctcagctgctgggcctgctgctgctgtggctgcgaggggctagatgtgataaaactcatacttgtcctccatgcccagcacctgaggcagcaggcgccccatccgtgttcctgtttccccctaagcccaaggacacactgatgatctcccgtacgccagaggtgacatgcgtggtggtggacgtgtctcacgaggaccccgaggtgaagttcaactggtacgtggatggcgtggaggtgcacaatgccaagaccaagcccagggaggagcagtacaacagcacctatcgcgtggtgtccgtgctgacagtgctgcaccaggactggctgaacggcaaggagtataagtgcaaggtgtccaataaggccctgccagcccccatcgagaagaccatcagcaaggcaaagggacagcctcgggagccacaggtgtgcaccctgccaccctctagagaggagatgacaaagaaccaggtgagcctgtggtgtctggtgaagggcttctacccttccgacatcgccgtggagtgggagtctaatggccagccagagaacaattacaagaccacacctccagtgctggactctgatggcagcttctttctgtattctaagctgaccgtggataagagcaggtggcagcagggcaacgtgttttcctgctctgtgatgcacgaggccctgcacaatcactacacacagaagagcctgtccctgtctcccggg

SEQ ID NO: 61 - DNA, 1110 bp, Artificial
  P-0668 Chain 1
atgtatcggatgcagctgctgtcttgtatcgctctgtcactggctctggtcactaattctaactgggtcaatgtcatttctgatctgaagaagatcgaggacctgatccagagcatgcacatcgatgccaccctgtacacagagtccgacgtgcacccatcttgcaaggtgaccgcaatgaagtgtttcctgctggagctgcaggtcatcagcctggagagcggcgacgcagatatccacgataccgtggagaacctgatcatcctggcaaacaattccctgagctccaacggaaatgtgacagagtctggatgcaaggagtgtgaggagctggaggagaagaacatcaaggagttcctgcagtcttttgtgcacatcgtgcagatgttcatcaatacatccggcggcggcggctccggcggcggcggctctggcggcggcggcagctgccccccttgtccagcccccgaggccgctggggcaccaagcgtgttcctgttccctccaaaaccaaaagatactctgatgattagccgtacgccagaggtgacatgcgtggtggtggacgtgagccacgaggaccccgaggtgaagtttaactggtacgtggacggcgtggaggtgcacaatgccaagacaaagcctagggaggagcagtacaattctacctatcgcgtggtgagcgtgctgacagtgctgcaccaggattggctgaacggcaaggagtataagtgcaaggtgtccaataaggccctgcctgccccaatcgagaagaccatctctaaggccaagggccagcccagagagcctcaggtgtacacactgcctccaagcagagacgagctgaccaagaaccaggtgtccctgacatgtctggtgaagggcttctatccctctgatatcgccgtggagtgggagagcaatggccagcctgagaacaattacaagaccacaccccctgtgctggacagcgatggctccttctttctgtattccaagctgaccgtggataagtctcggtggcagcagggcaacgtgttttcctgctctgtgatgcacgaagcactgcataaccactacacccagaagagcctgagcctgtcccccggg

SEQ ID NO: 62 - DNA, 1005 bp, Artificial
  P-0314 Chain 1
atggatatgcgggtgcctgctcagctgctgggcctgctgctgctgtggctgcgaggggctagatgtgataaaactcatacttgtcctccatgcccagcacctgaggcagcaggcgccccatccgtgttcctgtttccccctaagcccaaggacacactgatgatctcccgtacgccagaggtgacatgcgtggtggtggacgtgagccacgaggaccccgaggtgaagtttaactggtacgtggacggcgtggaggtgcacaatgccaagacaaagcctagggaggagcagtacaattctacctatcgcgtggtgagcgtgctgacagtgctgcaccaggattggctgaacggcaaggagtataagtgcaaggtgtccaataaggccctgcctgccccaatcgagaagaccatctctaaggccaagggccagcccagagagcctcaggtgtacacactgcctccaagcagagacgagctgaccaagaaccaggtgtccctgacatgtctggtgaagggcttctatccctctgatatcgccgtggagtgggagagcaatggccagcctgagaacaattacaagaccacaccccctgtgctggacagcgatggctccttctttctgtattccaagctgaccgtggataagtctcggtggcagcagggcaacgtgttttcctgctctgtgatgcacgaagcactgcataaccactacacccagaagagcctgagcctgtcccccgggggcggcggcggcagcggaggcggcggctccatcacctgtccaccccctatgagcgtggagcacgccgatatctgggtgaagagctactccctgtatagccgggagagatatatctgcaattccggctttaagcgcaaggccggcacctctagcctgacagagtgcgtgctgaacaaggccaccaatgtggcccactggacaaccccaagcctgaagtgtattagagaccctgccctggtgcatcagcggcctgctccccca

SEQ ID NO: 63 - DNA, 402 bp, Artificial
  P-0314 Chain 2
atgtaccggatgcagctgctgtcctgcatcgccctgtctctggccctggtgaccaactctaattgggtgaacgtgatcagcgacctgaagaagatcgaggatctgatccagtctatgcacatcgacgccaccctgtatacagagagcgatgtgcacccctcctgcaaggtgacagccatgaagtgtttcctgctggagctgcaggtcatcagcctggagagcggcgacgcagacatccacgataccgtggagaacctgatcatcctggccaataactccctgagctccaacggcaatgtgacagagtctggctgcaaggagtgtgaggagctggaggagaagaacatcaaggagttcctgcagagctttgtgcacatcgtgcagatgtttatcaatacctcc

SEQ ID NO: 64 - protein, 296 aa, Artificial
  Benchmark Chain1
ITCPPPMSVEHADIWVKSYSLYSRERYICNSGFKRKAGTSSLTECVLNKATNVAHWTTPSLKCIREPKSCDKTHTCPPCPAPELLGGPSVFLFPPKPKDTLMISRTPEVTCVVVDVSHEDPEVKFNWYVDGVEVHNAKTKPREEQYNSTYRVVSVLTVLHQDWLNGKEYKCKVSNKALPAPIEKTISKAKGQPREPQVYTLPPSRDELTKNQVSLTCLVKGFYPSDIAVEWESNGQPENNYKTTPPVLDSDGSFFLYSKLTVDKSRWQQGNVFSCSVMHEALHNHYTQKSLSLSPG

SEQ ID NO: 65 - protein, 114 aa, Artificial
  Benchmark Chain 2
NWVNVISDLKKIEDLIQSMHIDATLYTESDVHPSCKVTAMKCFLLELQVISLESGDASIHDTVENLIILANDSLSSNGNVTESGCKECEELEEKNIKEFLQSFVHIVQMFINTS